European Patent Application EP 4 162 941 A1, published April 12, 2023. Title: 可受微小RNA调控的分离的重组溶瘤痘病毒及其应用. Applicant: 杭州康万达医药科技有限公司. The sequence listing filed with the application follows.

SEQUENCE LISTING (38 sequences)

SEQ ID NO: 1 - DNA, 22 bp, 人（Homo sapiens）
acagtagtctgcacattggtta

SEQ ID NO: 2 - DNA, 30 bp, 人工序列（artificial sequence）
agtcctcgagctaatattgagaaattcatc

SEQ ID NO: 3 - DNA, 66 bp, 人工序列（artificial sequence）
ctgcacattggttattaagaagcatagtctggaacatcatatggatataaagggttaacctttgtc

SEQ ID NO: 4 - DNA, 59 bp, 人工序列（artificial sequence）
tggttaggacagtagtctgcacattggttaggacagtagtctgcacattggttattaag

SEQ ID NO: 5 - DNA, 61 bp, 人工序列（artificial sequence）
atgtgcagactactgtcctaaccaatgtgcagactactgtccaaaaattgaaaataaatac

SEQ ID NO: 6 - DNA, 32 bp, 人工序列（artificial sequence）
gatcaagatctttagtcctgctcctcggccac

SEQ ID NO: 7 - DNA, 36 bp, 人工序列（artificial sequence）
gatcaagatctttataaacttaacccattataaaac

SEQ ID NO: 8 - DNA, 33 bp, 人工序列（artificial sequence）
agtcggatccttgacagtcttgaacaattatac

SEQ ID NO: 9 - DNA, 28 bp, 人工序列（artificial sequence）
cccaagcttttagtcctgctcctcggcc

SEQ ID NO: 10 - DNA, 61 bp, 人工序列（artificial sequence）
ataacttcgtatagcatacattatacgaagttatctttataaacttaacccattataaaac

SEQ ID NO: 11 - DNA, 34 bp, 人工序列（artificial sequence）
ataacttcgtataatgtatgctatacgaagttat

SEQ ID NO: 12 - DNA, 20 bp, 人工序列（artificial sequence）
cgcgtatttgggatcagatg

SEQ ID NO: 13 - DNA, 21 bp, 人工序列（artificial sequence）
caaaggttcttgagggttgtg

SEQ ID NO: 14 - DNA, 20 bp, 人工序列（artificial sequence）
gttgatcggcacgtaagagg

SEQ ID NO: 15 - DNA, 23 bp, 人工序列（artificial sequence）
gtcacagaaaccatgccgtgtag

SEQ ID NO: 16 - DNA, 19 bp, 人工序列（artificial sequence）
ggagcttccagggggaaac

SEQ ID NO: 17 - DNA, 19 bp, 人工序列（artificial sequence）
gacctcagcgtcgtagtgg

SEQ ID NO: 18 - DNA, 21 bp, 人工序列（artificial sequence）
ccaattaatgcaccgaacatc

SEQ ID NO: 19 - DNA, 21 bp, 人工序列（artificial sequence）
atgaattggaggagatggtgg

SEQ ID NO: 20 - DNA, 20 bp, 人工序列（artificial sequence）
taatacgactcactataggg

SEQ ID NO: 21 - DNA, 24 bp, 人工序列（artificial sequence）
atcgcattttctaacgtgatggat

SEQ ID NO: 22 - DNA, 23 bp, 人工序列（artificial sequence）
tatctaacgacacaacatccatt

SEQ ID NO: 23 - DNA, 20 bp, 人工序列（artificial sequence）
gcacggtaaggaagtagatc

SEQ ID NO: 24 - DNA, 22 bp, 人工序列（artificial sequence）
cagtacacggtcctcagcataa

SEQ ID NO: 25 - DNA, 18 bp, 人工序列（artificial sequence）
cagggaaacggatgtata

SEQ ID NO: 26 - DNA, 22 bp, 人工序列（artificial sequence）
tgtgttacagaatcatataagg

SEQ ID NO: 27 - DNA, 52 bp, 人工序列（artificial sequence）
gtcgtatccagtgcagggtccgaggtattcgcactggatacgacaaaatatg

SEQ ID NO: 28 - DNA, 19 bp, 人工序列（artificial sequence）
ctcgcttcggcagcacata

SEQ ID NO: 29 - DNA, 19 bp, 人工序列（artificial sequence）
cgcagggtccgaggtattc

SEQ ID NO: 30 - DNA, 51 bp, 人工序列（artificial sequence）
gtcgtatccagtgcagggtccgaggtattcgcactggatacgactaaccaa

SEQ ID NO: 31 - DNA, 23 bp, 人工序列（artificial sequence）
gccgacagtagtctgcacattgg

SEQ ID NO: 32 - DNA, 19 bp, 人工序列（artificial sequence）
cgcagggtccgaggtattc

SEQ ID NO: 33 - DNA, 28 bp, 人工序列（artificial sequence）
ccgctcgaggctggcgtttttccatagg

SEQ ID NO: 34 - DNA, 33 bp, 人工序列（artificial sequence）
cgcggatcccggtctggttataggtacattgag

SEQ ID NO: 35 - DNA, 261 bp, 人工序列（artificial sequence）
caatttaacacaaccctcaagaacctttgtatttattttcaatttttataacttcgtataatgtatgctatacgaagttatggacagtagtctgcacattggttaggacagtagtctgcacattggttaggacagtagtctgcacattggttaggacagtagtctgcacattggttattaagaagcatagtctggaacatcatatggatataaagggttaacctttgtcacatcgatcgcgtatttgggatcagatggtac

SEQ ID NO: 36 - DNA, 44 bp, 人工序列（artificial sequence）
gtcgtatccagtgcagggtccgaggtattcgcactggatacgac

SEQ ID NO: 37 - DNA, 69 bp, 人工序列（artificial sequence）
gatccgacagtagtctgcacattggttattcaagagataaccaatgcagactactgtcttttttgaatt

SEQ ID NO: 38 - DNA, 65 bp, 人工序列（artificial sequence）
gatccgttctccgaacgtgtcacgtttcaagagaacgtgacacgttcggagaacttttttgaatt